European Patent Application EP 4 656 731 A1, published December 3, 2025. Title: Verfahren zur Herstellung von Galactarsäure. Applicant: Annikki GmbH. Application EP. The sequence listing filed with the application follows.

SEQUENCE LISTING (4 sequences)

SEQ ID NO: 1 - DNA, 1356 bp, Carnobacterium divergens
  source 1..1356: mol_type = genomic DNA
atgaaagtagtagtagtaggctgtacacatgcaggaacagcggcagttaagacgattttaaatgaacatccagatgcatcagtatcagtatatgagcgtaatgacaatgtctcatttctatcttgtgggattgcgttgtatgttggtggagttgtgaaagatcctgcaggtttgttttattcaagtccagaagaacttgcatcaatgggcgcgaaaattaacatggaacacaatgtgaaaaatatagataatgagaataaggtcgtagtaattgagaatttaaaaacaggcgaaacatttgaagaaagctatgataagttggtaatgacaactggatcatggccaattattcctccaattgatggaatcaatagtgaaaatattcttttgtgtaaaaactataaccaagcaaatgaaattattaaagaatcaaaaaatgctaaaaagattgtcattgttggtggtggctatattggaattgaattagttgaggcatttgcagaatctggcaagcaagtgacgctagttgatggattagatcgtattttaaacaaatatttagatgctgaattcacttctgttttagagcatgatttacaagaaagaggcgttacgctagctttaaaccaaaccgtcgagaaatttgttgccaatgaatcaggtgctgtgacagctgtgaaaacaccagttggagaatatgaggctgatttagttattttatgtgttggatttaaaccaaatactgatttgttgaaggataaagtagagatgttgccaaatggtgccatcgtagtggatgaatatatgagaacaagcgatgaagcgatttttgctgctggcgatagttgcgcggttcattataatccaactggaggctctgcgtatattccgttagctacaaatgcagttagaatgggagctttagttgggaaaaatattgtttctccaacagttaaatatcgtggcacgcaagcaacttctggtttatatttatttggttttaatataggttcaaccggattgactgaaaatagcgctcctcattttggcgtagaggttcgttcagtagttgtagaagataattatcgtccagagtttatgccgacaacagagaaagtaacgatgaaattagtttatgaagtaggaacgaatcggattgttggaggtcaaatcatgtcaaaatatgatgtgacacaatctgccaatacgttatctttatgtgttcaaaataaaatgacgattgaggatttggcttatgtagatttcttcttccaacctcactttgatcgtccttggaactatttaaatattttagcgcaagcagctgttgagcaagagcgtaaactagcaaaataa

SEQ ID NO: 2 - protein, 451 aa, Carnobacterium divergens
MKVVVVGCTHAGTAAVKTILNEHPDASVSVYERNDNVSFLSCGIALYVGGVVKDPAGLFYSSPEELASMGAKINMEHNVKNIDNENKVVVIENLKTGETFEESYDKLVMTTGSWPIIPPIDGINSENILLCKNYNQANEIIKESKNAKKIVIVGGGYIGIELVEAFAESGKQVTLVDGLDRILNKYLDAEFTSVLEHDLQERGVTLALNQTVEKFVANESGAVTAVKTPVGEYEADLVILCVGFKPNTDLLKDKVEMLPNGAIVVDEYMRTSDEAIFAAGDSCAVHYNPTGGSAYIPLATNAVRMGALVGKNIVSPTVKYRGTQATSGLYLFGFNIGSTGLTENSAPHFGVEVRSVVVEDNYRPEFMPTTEKVTMKLVYEVGTNRIVGGQIMSKYDVTQSANTLSLCVQNKMTIEDLAYVDFFFQPHFDRPWNYLNILAQAAVEQERKLAK

SEQ ID NO: 3 - DNA, 1374 bp, Streptococcus mutans
  source 1..1374: mol_type = genomic DNA
atgagcaaaattgttatcgtgggtgcaaatcatgcaggcaccgcagcaattaataccattctggataattatggcagcgaaaatgaagtggttgtgtttgatcagaatagcaacattagctttctgggttgtggtatggcactgtggattggtaaacaaattagcggtccgcagggtctgttttatgcagataaagaaagcctggaagcaaaaggtgccaaaatctatatggaaagtccggttaccgccattgattatgatgcaaaacgtgttaccgcactggttaatggtcaagaacatgttgaaagctacgagaaactgattctggcaaccggtagcaccccgattctgcctccgattaaaggtgcagccattaaagaaggtagtcgcgattttgaagcaaccctgaaaaatctgcagttcgtgaaactgtatcagaatgccgaagatgtgattaacaaactgcaggataaaagccagaatctgaatcgtattgcagttgttggtgcaggttatattggtgttgaactggcagaagcatttaaacgtctgggtaaagaagtgattctgattgacgttgttgatacctgtctggcaggttattatgatcaggatctgagcgaaatgatgcgtcagaatctggaagatcatggtatcgaactggcatttggtgaaaccgttaaagcaattgaaggtgatggtaaagtggaacgtattgttaccgataaagcaagccatgatgtggatatggttattctggcagttggttttcgtccgaatacagcactgggtaatgcaaaactgaaaacctttcgtaatggtgcctttctggtggataaaaaacaagaaaccagcatcccggatgtttatgcaattggtgattgtgcaaccgtgtatgataatgccattaacgacaccaactatattgcactggcaagcaatgcactgcgtagcggtattgttgcaggtcataatgcagccggtcataaactggaaagtctgggtgttcagggtagcaatggtatttcaatttttggcctgaatatggttagcaccggtctgacccaagaaaaagccaaacgttttggttataatccggaagttaccgcctttaccgattttcagaaagccagctttatcgagcatgataactatccggttacgctgaaaattgtgtatgacaaagatagccgtctggttctgggtgcacagatggccagcaaagaagatatgagcatgggtattcacatgtttagcctggccattcaagagaaagttaccattgaacgtctggccctgctggattatttctttctgccgcattttaatcagccgtacaactatatgaccaaagcagcactgaaagccaaataa

SEQ ID NO: 4 - protein, 457 aa, Streptococcus mutans
MSKIVIVGANHAGTAAINTILDNYGSENEVVVFDQNSNISFLGCGMALWIGKQISGPQGLFYADKESLEAKGAKIYMESPVTAIDYDAKRVTALVNGQEHVESYEKLILATGSTPILPPIKGAAIKEGSRDFEATLKNLQFVKLYQNAEDVINKLQDKSQNLNRIAVVGAGYIGVELAEAFKRLGKEVILIDVVDTCLAGYYDQDLSEMMRQNLEDHGIELAFGETVKAIEGDGKVERIVTDKASHDVDMVILAVGFRPNTALGNAKLKTFRNGAFLVDKKQETSIPDVYAIGDCATVYDNAINDTNYIALASNALRSGIVAGHNAAGHKLESLGVQGSNGISIFGLNMVSTGLTQEKAKRFGYNPEVTAFTDFQKASFIEHDNYPVTLKIVYDKDSRLVLGAQMASKEDMSMGIHMFSLAIQEKVTIERLALLDYFFLPHFNQPYNYMTKAALKAK